European Patent Application EP 4 509 519 A1, published February 19, 2025. Title: EXOSOME COMPOSITION CONTAINING GANODERMA IMMUNOMODULATORY PROTEIN AND USES THEREOF. Applicant: MYCOMAGIC BIOTECHNOLOGY CO., LTD. Application US. The sequence listing filed with the application follows.

SEQUENCE LISTING (8 sequences)

SEQ ID NO: 1 - protein, 6 aa, synthetic construct
LAWNVK

SEQ ID NO: 2 - protein, 10 aa, synthetic construct
DLGVRPSYAV

SEQ ID NO: 3 - protein, 111 aa, synthetic construct
MSDTALIFTLAWNVKQLAFDYTPNWGRGRPSSFIDTVTFPTVLTDKAYTYRVVVSGKDLGVRPSYAVESDGSQKINFLEYNSGYGIADTNTIQVYVIDPDTGNNFIVAQWN

SEQ ID NO: 4 - protein, 140 aa, synthetic construct
EAEAEFMSDTALIFTLAWNVKQLAFDYTPNWGRGRPSSFIDTVTFPTVLTDKAYTYRVVVSGKDLGVRPSYAVESDGSQKINFLEYNSGYGIADTNTIQVYVIDPDTGNNFIVAQWNYLEQKLISEEDLNSAVDHHHHHH

SEQ ID NO: 5 - DNA, 23 bp, synthetic construct
  source 1..23: mol_type = other DNA
gaattcatgtccgacactgcctt

SEQ ID NO: 6 - DNA, 22 bp, synthetic construct
  source 1..22: mol_type = other DNA
gttccactgggcaacaatgaaa

SEQ ID NO: 7 - DNA, 19 bp, synthetic construct
  source 1..19: mol_type = other DNA
tccgtaggtgaacctgcgg

SEQ ID NO: 8 - DNA, 20 bp, synthetic construct
  source 1..20: mol_type = other DNA
tcctccgcttattgatatgc